European Patent Specification EP 2 812 442 B9, published February 15, 2023. Title: A METHOD FOR CHEMOENZYMATIC GLYCOENGINEERING OF ANTIBODIES AND FC FRAGMENTS THEREOF. Applicant: University of Maryland, Baltimore Wang, Lai-Xi Huang, Wei. Application EP13746579.5. The sequence listing filed with the application follows.

SEQUENCE LISTING (5 sequences)

SEQ ID NO: 1 - protein, 995 aa, Streptococcus pyogenes
MDKHLLVKRTLGCVCAATLMGAALATHHDSLNTVKAEEKTVQVQKGLPSIDSLHYLSENSKKEFKEELSKAGQESQKVKEILAKAQQADKQAQELAKMKIPEKIPMKPLHGPLYGGYFRTWHDKTSDPTEKDKVNSMGELPKEVDLAFIFHDWTKDYSLFWKELATKHVPKLNKQGTRVIRTIPWRFLAGGDNSGIAEDTSKYPNTPEGNKALAKAIVDEYVYKYNLDGLDVDVEHDSIPKVDKKEDTAGVERSIQVFEEIGKLIGPKGVDKSRLFIMDSTYMADKNPLIERGAPYINLLLVQVYGSQGEKGGWEPVSNRPEKTMEERWQGYSKYIRPEQYMIGFSFYEENAQEGNLWYDINSRKDEDKANGINTDITGTRAERYARWQPKTGGVKGGIFSYAIDRDGVAHQPKKYAKQKEFKDATDNIFHSDYSVSKALKTVMLKDKSYDLIDEKDFPDKALREAVMAQVGTRKGDLERFNGTLRLDNPAIQSLEGLNKFKKLAQLDLIGLSRITKLDRSVLPANMKPGKDTLETVLETYKKDNKEEPATIPPVSLKVSGLTGLKELDLSGFDRETLAGLDAATLTSLEKVDISGNKLDLAPGTENRQIFDTMLSTISNHVGSNEQTVKFDKQKPTGHYPDTYGKTSLRLPVANEKVDLQSQLLFGTVTNQGTLINSEADYKAYQNHKIAGRSFVDSNYHYNNFKVSYENYTVKVTDSTLGTTTDKTLATDKEETYKVDFFSPADKTKAVHTAKVIVGDEKTMMVNLAEGATVIGGSADPVNARKVFDGQLGSETDNISLGWDSKQSIIFKLKEDGLIKHWRFFNDSARNPETTNKPIQEASLQIFNIKDYNLDNLLENPNKFDDEKYWITVDTYSAQGERATAFSNTLNNITSKYWRVVFDTKGDRYSSPVVPELQILGYPLPNADTIMKTVTTAKELSQQKDKFSQKMLDELKIKEMALETSLNSKIFDVTAINANAGVLKDCIEKRQLLKK

SEQ ID NO: 2 - protein, 995 aa, Artificial Sequence
  Synthetic construct
MDKHLLVKRTLGCVCAATLMGAALATHHDSLNTVKAEEKTVQVQKGLPSIDSLHYLSENSKKEFKEELSKAGQESQKVKEILAKAQQADKQAQELAKMKIPEKIPMKPLHGPLYGGYFRTWHDKTSDPTEKDKVNSMGELPKEVDLAFIFHDWTKDYSLFWKELATKHVPKLNKQGTRVIRTIPWRFLAGGDNSGIAEDTSKYPNTPEGNKALAKAIVDEYVYKYNLDGLDVQVEHDSIPKVDKKEDTAGVERSIQVFEEIGKLIGPKGVDKSRLFIMDSTYMADKNPLIERGAPYINLLLVQVYGSQGEKGGWEPVSNRPEKTMEERWQGYSKYIRPEQYMIGFSFYEENAQEGNLWYDINSRKDEDKANGINTDITGTRAERYARWQPKTGGVKGGIFSYAIDRDGVAHQPKKYAKQKEFKDATDNIFHSDYSVSKALKTVMLKDKSYDLIDEKDFPDKALREAVMAQVGTRKGDLERFNGTLRLDNPAIQSLEGLNKFKKLAQLDLIGLSRITKLDRSVLPANMKPGKDTLETVLETYKKDNKEEPATIPPVSLKVSGLTGLKELDLSGFDRETLAGLDAATLTSLEKVDISGNKLDLAPGTENRQIFDTMLSTISNHVGSNEQTVKFDKQKPTGHYPDTYGKTSLRLPVANEKVDLQSQLLFGTVTNQGTLINSEADYKAYQNHKIAGRSFVDSNYHYNNFKVSYENYTVKVTDSTLGTTTDKTLATDKEETYKVDFFSPADKTKAVHTAKVIVGDEKTMMVNLAEGATVIGGSADPVNARKVFDGQLGSETDNISLGWDSKQSIIFKLKEDGLIKHWRFFNDSARNPETTNKPIQEASLQIFNIKDYNLDNLLENPNKFDDEKYWITVDTYSAQGERATAFSNTLNNITSKYWRVVFDTKGDRYSSPVVPELQILGYPLPNADTIMKTVTTAKELSQQKDKFSQKMLDELKIKEMALETSLNSKIFDVTAINANAGVLKDCIEKRQLLKK

SEQ ID NO: 3 - protein, 995 aa, Artificial Sequence
  Synthetic Construct
MDKHLLVKRTLGCVCAATLMGAALATHHDSLNTVKAEEKTVQVQKGLPSIDSLHYLSENSKKEFKEELSKAGQESQKVKEILAKAQQADKQAQELAKMKIPEKIPMKPLHGPLYGGYFRTWHDKTSDPTEKDKVNSMGELPKEVDLAFIFHDWTKDYSLFWKELATKHVPKLNKQGTRVIRTIPWRFLAGGDNSGIAEDTSKYPNTPEGNKALAKAIVDEYVYKYNLDGLDVAVEHDSIPKVDKKEDTAGVERSIQVFEEIGKLIGPKGVDKSRLFIMDSTYMADKNPLIERGAPYINLLLVQVYGSQGEKGGWEPVSNRPEKTMEERWQGYSKYIRPEQYMIGFSFYEENAQEGNLWYDINSRKDEDKANGINTDITGTRAERYARWQPKTGGVKGGIFSYAIDRDGVAHQPKKYAKQKEFKDATDNIFHSDYSVSKALKTVMLKDKSYDLIDEKDFPDKALREAVMAQVGTRKGDLERFNGTLRLDNPAIQSLEGLNKFKKLAQLDLIGLSRITKLDRSVLPANMKPGKDTLETVLETYKKDNKEEPATIPPVSLKVSGLTGLKELDLSGFDRETLAGLDAATLTSLEKVDISGNKLDLAPGTENRQIFDTMLSTISNHVGSNEQTVKFDKQKPTGHYPDTYGKTSLRLPVANEKVDLQSQLLFGTVTNQGTLINSEADYKAYQNHKIAGRSFVDSNYHYNNFKVSYENYTVKVTDSTLGTTTDKTLATDKEETYKVDFFSPADKTKAVHTAKVIVGDEKTMMVNLAEGATVIGGSADPVNARKVFDGQLGSETDNISLGWDSKQSIIFKLKEDGLIKHWRFFNDSARNPETTNKPIQEASLQIFNIKDYNLDNLLENPNKFDDEKYWITVDTYSAQGERATAFSNTLNNITSKYWRVVFDTKGDRYSSPVVPELQILGYPLPNADTIMKTVTTAKELSQQKDKFSQKMLDELKIKEMALETSLNSKIFDVTAINANAGVLKDCIEKRQLLKK

SEQ ID NO: 4 - protein, 60 aa, Artificial Sequence
  Sysnthetic Construct
RTIPWRFLAGGDNSGIAEDTSKYPNTPEGNKALAKAIVDEYVYKYNLDGLDVDVEHDSIP

SEQ ID NO: 5 - protein, 47 aa, Artificial Sequence
  Synthetic construct
QNIDDDVSWQSSKPGGFASAAAYGDAIKSIVIDKWKLDGISLDIEHS